European Patent Specification EP 3 936 514 B1, published May 24, 2023. Title: 3'3' CYCLIC DINUCLEOTIDES WITH AN ALKENYLENE. Applicant: Institute of Organic Chemistry and Biochemistry ASCR, v. v. i. The sequence listing filed with the application follows.

SEQUENCE LISTING (12 sequences)

SEQ ID NO: 1 - DNA, 75 bp, Artificial
  Synthetic oligonucleotide
aaagatcttggaaagtgaaaccttggaaaacgaaactggacaaagggaaactgcagaaactgaaacaaagcttaa

SEQ ID NO: 2 - DNA, 75 bp, Artificial
  Synthetic oligonucleotide
ttaagctttgtttcagtttctgcagtttccctttgtccagtttcgttttccaaggtttcactttccaagatcttt

SEQ ID NO: 3 - DNA, 20 bp, Artificial
  Forward primer
tgcttgctcaactctacgtc

SEQ ID NO: 4 - DNA, 20 bp, Artificial
  Reverse primer
gtggtttgtccaaactcatc

SEQ ID NO: 5 - DNA, 31 bp, Artificial
  Forward primer
gtgggatccgccccagctgagatctctgcag

SEQ ID NO: 6 - DNA, 38 bp, Artificial
  Reverse primer
tatgcggccgcctattacacagtaacctcttccttttc

SEQ ID NO: 7 - DNA, 330 bp, Artificial
  8-His-SUMO
atgtcgcatcaccatcatcatcaccaccatgggatgtcggactcagaagtcaatcaagaagctaagccagaggtcaagccagaagtcaagcctgagactcacatcaatttaaaggtgtccgatggatcttcagagatcttcttcaagatcaaaaagaccactcctttaagaaggctgatggaagcgttcgctaaaagacagggtaaggaaatggactccttaagattcttgtacgacggtattagaattcaagctgatcagacccctgaagatttggacatggaggataacgatattattgaggctcaccgcgaacagattggtggatcc

SEQ ID NO: 8 - protein, 110 aa, Artificial
  8-His-SUMO
MSHHHHHHHHGMSDSEVNQEAKPEVKPEVKPETHINLKVSDGSSEIFFKIKKTTPLRRLMEAFAKRQGKEMDSLRFLYDGIRIQADQTPEDLDMEDNDIIEAHREQIGGS

SEQ ID NO: 9 - protein, 204 aa, Artificial
  truncated WT STING
APAEISAVCEKGNFNVAHGLAWSYYIGYLRLILPELQARIRTYNQHYNNLLRGAVSQRLYILLPLDCGVPDNLSMADPNIRFLDKLPQQTGDRAGIKDRVYSNSIYELLENGQRAGTCVLEYATPLQTLFAMSQYSQAGFSREDRLEQAKLFCRTLEDILADAPESQNNCRLIAYQEPADDSSFSLSQEVLRHLRQEEKEEVTV

SEQ ID NO: 10 - protein, 204 aa, Artificial
  truncated AQ STING
APAEISAVCEKGNFNVAHGLAWSYYIGYLRLILPELQARIRTYNQHYNNLLRGAVSQRLYILLPLDCGVPDNLSMADPNIRFLDKLPQQTADRAGIKDRVYSNSIYELLENGQRAGTCVLEYATPLQTLFAMSQYSQAGFSREDRLEQAKLFCQTLEDILADAPESQNNCRLIAYQEPADDSSFSLSQEVLRHLRQEEKEEVTV

SEQ ID NO: 11 - protein, 392 aa, Artificial
  murine cGAS
MKYLLPTAAAGLLLLAAQPAMAMPDKLKKVLDKLRLKRKDISEAAETVNKVVERLLRRMQKRESEFKGVEQLNTGSYYEHVKISAPNEFDVMFKLEVPRIELQEYYETGAFYLVKFKRIPRGNPLSHFLEGEVLSATKMLSKFRKIIKEEVKEIKDIDVSVEKEKPGSPAVTLLIRNPEEISVDIILALESKGSWPISTKEGLPIQGWLGTKVRTNLRREPFYLVPKNAKDGNSFQGETWRLSFSHTEKYILNNHGIEKTCCESSGAKCCRKECLKLMKYLLEQLKKEFQELDAFCSYHVKTAIFHMWTQDPQDSQWDPRNLSSCFDKLLAFFLECLRTEKLDHYFIPKFNLFSQELIDRKSKEFLSKKIEYERNNGFPIFDKLLEHHHHHH

SEQ ID NO: 12 - protein, 365 aa, Artificial
  BMB171
MEENKQRVKSMINILQLVAPGTPLREGIDNVLRAQTGGLIVLGYNEQIKSIVDGGFHINCAFSPASLYELAKMDGALILNETGSKILIANAQLVPDSSIDSIETGMRHRTAERVAKQTGSLVVAISQRRNVITLYQGNLRYTLKDIGVILTKANQAIQTLEKYKAVWNDGITNLGILEFEEVVTMSEVVHVLHSVEMVLRIKNEILSYIHELGTEGRLIRLQLTELLADLEAEAALLIKDYHQEKTQDHHQILKKLQDLANTQLLEDSDLVKLLGYPGQTSLEESVTPRGYRITSKISRVPPLIIENLINRFKTLQGVCRATINELDDVEGIGEVRAKKIREGLKRIQEHLYMSRHNLEHHHHHH